European Patent Application EP 4 778 535 A1, published July 22, 2026. Title: 药物组合及用途. Applicant: 中山康方生物医药有限公司. The sequence listing filed with the application follows.

SEQUENCE LISTING (92 sequences)

SEQ ID NO: 1 - protein, 8 aa, synthetic construct
  source 1..8: note = HCDR1
GFAFSSYD

SEQ ID NO: 2 - protein, 8 aa, synthetic construct
  source 1..8: note = HCDR2
ISGGGRYT

SEQ ID NO: 3 - protein, 11 aa, synthetic construct
  source 1..11: note = HCDR3
ANRYGEAWFAY

SEQ ID NO: 4 - protein, 6 aa, synthetic construct
  source 1..6: note = LCDR1
QDINTY

SEQ ID NO: 5 - skipped

SEQ ID NO: 6 - protein, 9 aa, synthetic construct
  source 1..9: note = LCDR3
LQYDEFPLT

SEQ ID NO: 7 - protein, 8 aa, synthetic construct
  source 1..8: note = HCDR1
GYTFTNYG

SEQ ID NO: 8 - protein, 8 aa, synthetic construct
  source 1..8: note = HCDR2
INTYTGEP

SEQ ID NO: 9 - protein, 16 aa, synthetic construct
  source 1..16: note = HCDR3
AKYPHYYGSSHWYFDV

SEQ ID NO: 10 - protein, 6 aa, synthetic construct
  source 1..6: note = LCDR1
QDISNY

SEQ ID NO: 11 - skipped

SEQ ID NO: 12 - protein, 9 aa, synthetic construct
  source 1..9: note = LCDR3
QQYSTVPWT

SEQ ID NO: 13 - protein, 9 aa, synthetic construct
  source 1..9: note = HCDR1
GHSFTSDYA

SEQ ID NO: 14 - protein, 7 aa, synthetic construct
  source 1..7: note = HCDR2
ISYSDST

SEQ ID NO: 15 - protein, 14 aa, synthetic construct
  source 1..14: note = HCDR3
ARLDYGNYGGAMDY

SEQ ID NO: 16 - protein, 6 aa, synthetic construct
  source 1..6: note = LCDR1
QHVSTA

SEQ ID NO: 17 - skipped

SEQ ID NO: 18 - protein, 9 aa, synthetic construct
  source 1..9: note = LCDR3
QQHYITPWT

SEQ ID NO: 19 - DNA, 354 bp, synthetic construct
  source 1..354: mol_type = other DNA; note = nucleic acid encoding VH of 14C12
gaggtcaaactggtggagagcggcggcgggctggtgaagcccggcgggtcactgaaactgagctgcgccgcttccggcttcgcctttagctcctacgacatgtcatgggtgaggcagacccctgagaagcgcctggaatgggtcgctactatcagcggaggcgggcgatacacctactatcctgactctgtcaaagggagattcacaattagtcgggataacgccagaaatactctgtatctgcagatgtctagtctgcggtccgaggatacagctctgtactattgtgcaaaccggtacggcgaagcatggtttgcctattggggacagggcaccctggtgacagtctctgcc

SEQ ID NO: 20 - protein, 118 aa, synthetic construct
  source 1..118: note = amino acid sequence of VH of 14C12
EVKLVESGGGLVKPGGSLKLSCAASGFAFSSYDMSWVRQTPEKRLEWVATISGGGRYTYYPDSVKGRFTISRDNARNTLYLQMSSLRSEDTALYYCANRYGEAWFAYWGQGTLVTVSA

SEQ ID NO: 21 - DNA, 321 bp, synthetic construct
  source 1..321: mol_type = other DNA; note = nucleic acid encoding VL of 14C12
gacattaagatgacacagtccccttcctcaatgtacgctagcctgggcgagcgagtgaccttcacatgcaaagcatcccaggacatcaacacatacctgtcttggtttcagcagaagccaggcaaaagccccaagaccctgatctaccgggccaatagactggtggacggggtccccagcagattctccggatctggcagtgggcaggattactccctgaccatcagctccctggagtatgaagacatgggcatctactattgcctgcagtatgatgagttccctctgacctttggagcaggcacaaaactggaactgaag

SEQ ID NO: 22 - protein, 107 aa, synthetic construct
  source 1..107: note = amino acid sequence of VL of 14C12
DIKMTQSPSSMYASLGERVTFTCKASQDINTYLSWFQQKPGKSPKTLIYRANRLVDGVPSRFSGSGSGQDYSLTISSLEYEDMGIYYCLQYDEFPLTFGAGTKLELK

SEQ ID NO: 23 - DNA, 354 bp, synthetic construct
  source 1..354: mol_type = other DNA; note = nucleic acid encoding VH of 14C12H1L1
gaagtgcagctggtcgagtctgggggagggctggtgcagcccggcgggtcactgcgactgagctgcgcagcttccggattcgcctttagctcctacgacatgtcctgggtgcgacaggcaccaggaaagggactggattgggtcgctactatctcaggaggcgggagatacacctactatcctgacagcgtcaagggccggttcacaatctctagagataacagtaagaacaatctgtatctgcagatgaacagcctgagggctgaggacaccgcactgtactattgtgccaaccgctacggggaagcatggtttgcctattgggggcagggaaccctggtgacagtctctagt

SEQ ID NO: 24 - protein, 118 aa, synthetic construct
  source 1..118: note = amino acid sequence of VH of 14C12H1L1
EVQLVESGGGLVQPGGSLRLSCAASGFAFSSYDMSWVRQAPGKGLDWVATISGGGRYTYYPDSVKGRFTISRDNSKNNLYLQMNSLRAEDTALYYCANRYGEAWFAYWGQGTLVTVSS

SEQ ID NO: 25 - DNA, 321 bp, synthetic construct
  source 1..321: mol_type = other DNA; note = nucleic acid encoding VL of 14C12H1L1
gacattcagatgactcagagcccctcctccatgtccgcctctgtgggcgacagggtcaccttcacatgccgcgctagtcaggatatcaacacctacctgagctggtttcagcagaagccagggaaaagccccaagacactgatctaccgggctaatagactggtgtctggagtcccaagtcggttcagtggctcagggagcggacaggactacactctgaccatcagctccctgcagcctgaggacatggcaacctactattgcctgcagtatgatgagttcccactgacctttggcgccgggacaaaactggagctgaag

SEQ ID NO: 26 - protein, 107 aa, synthetic construct
  source 1..107: note = amino acid sequence of VL of 14C12H1L1
DIQMTQSPSSMSASVGDRVTFTCRASQDINTYLSWFQQKPGKSPKTLIYRANRLVSGVPSRFSGSGSGQDYTLTISSLQPEDMATYYCLQYDEFPLTFGAGTKLELK

SEQ ID NO: 27 - DNA, 1344 bp, synthetic construct
  source 1..1344: mol_type = other DNA; note = nucleic acid encoding HC of 14C12H1L1
gaagtgcagctggtcgagtctgggggagggctggtgcagcccggcgggtcactgcgactgagctgcgcagcttccggattcgcctttagctcctacgacatgtcctgggtgcgacaggcaccaggaaagggactggattgggtcgctactatctcaggaggcgggagatacacctactatcctgacagcgtcaagggccggttcacaatctctagagataacagtaagaacaatctgtatctgcagatgaacagcctgagggctgaggacaccgcactgtactattgtgccaaccgctacggggaagcatggtttgcctattgggggcagggaaccctggtgacagtctctagtgccagcaccaaaggacctagcgtgtttcctctcgccccctcctccaaaagcaccagcggaggaaccgctgctctcggatgtctggtgaaggactacttccctgaacccgtcaccgtgagctggaatagcggcgctctgacaagcggagtccatacattccctgctgtgctgcaaagcagcggactctattccctgtccagcgtcgtcacagtgcccagcagcagcctgggcacccagacctacatctgtaacgtcaaccacaagccctccaacaccaaggtggacaagaaagtggagcccaaatcctgcgacaagacacacacctgtcccccctgtcctgctcccgaactcctcggaggccctagcgtcttcctctttcctcccaaacccaaggacaccctcatgatcagcagaacccctgaagtcacctgtgtcgtcgtggatgtcagccatgaggaccccgaggtgaaattcaactggtatgtcgatggcgtcgaggtgcacaacgccaaaaccaagcccagggaggaacagtacaactccacctacagggtggtgtccgtgctgacagtcctccaccaggactggctgaacggcaaggagtacaagtgcaaggtgtccaacaaggctctccctgcccccattgagaagaccatcagcaaggccaaaggccaacccagggagccccaggtctatacactgcctccctccagggacgaactcaccaagaaccaggtgtccctgacctgcctggtcaagggcttttatcccagcgacatcgccgtcgagtgggagtccaacggacagcccgagaataactacaagaccacccctcctgtcctcgactccgacggctccttcttcctgtacagcaagctgaccgtggacaaaagcaggtggcagcagggaaacgtgttctcctgcagcgtgatgcacgaagccctccacaaccactacacccagaaaagcctgtccctgagccccggcaaa

SEQ ID NO: 28 - protein, 448 aa, synthetic construct
  source 1..448: note = amino acid sequence of HC of 14C12H1L1
EVQLVESGGGLVQPGGSLRLSCAASGFAFSSYDMSWVRQAPGKGLDWVATISGGGRYTYYPDSVKGRFTISRDNSKNNLYLQMNSLRAEDTALYYCANRYGEAWFAYWGQGTLVTVSSASTKGPSVFPLAPSSKSTSGGTAALGCLVKDYFPEPVTVSWNSGALTSGVHTFPAVLQSSGLYSLSSVVTVPSSSLGTQTYICNVNHKPSNTKVDKKVEPKSCDKTHTCPPCPAPELLGGPSVFLFPPKPKDTLMISRTPEVTCVVVDVSHEDPEVKFNWYVDGVEVHNAKTKPREEQYNSTYRVVSVLTVLHQDWLNGKEYKCKVSNKALPAPIEKTISKAKGQPREPQVYTLPPSRDELTKNQVSLTCLVKGFYPSDIAVEWESNGQPENNYKTTPPVLDSDGSFFLYSKLTVDKSRWQQGNVFSCSVMHEALHNHYTQKSLSLSPGK

SEQ ID NO: 29 - DNA, 642 bp, synthetic construct
  source 1..642: mol_type = other DNA; note = nucleic acid encoding LC of 14C12H1L1
gacattcagatgactcagagcccctcctccatgtccgcctctgtgggcgacagggtcaccttcacatgccgcgctagtcaggatatcaacacctacctgagctggtttcagcagaagccagggaaaagccccaagacactgatctaccgggctaatagactggtgtctggagtcccaagtcggttcagtggctcagggagcggacaggactacactctgaccatcagctccctgcagcctgaggacatggcaacctactattgcctgcagtatgatgagttcccactgacctttggcgccgggacaaaactggagctgaagcgaactgtggccgctccctccgtcttcatttttcccccttctgacgaacagctgaaatcaggcacagccagcgtggtctgtctgctgaacaatttctaccctagagaggcaaaagtgcagtggaaggtcgataacgccctgcagtccggcaacagccaggagagtgtgactgaacaggactcaaaagatagcacctattccctgtctagtacactgactctgtccaaggctgattacgagaagcacaaagtgtatgcatgcgaagtgacacatcagggactgtcaagccccgtgactaagtcttttaaccggggcgaatgt

SEQ ID NO: 30 - protein, 214 aa, synthetic construct
  source 1..214: note = amino acid sequence of LC of 14C12H1L1
DIQMTQSPSSMSASVGDRVTFTCRASQDINTYLSWFQQKPGKSPKTLIYRANRLVSGVPSRFSGSGSGQDYTLTISSLQPEDMATYYCLQYDEFPLTFGAGTKLELKRTVAAPSVFIFPPSDEQLKSGTASVVCLLNNFYPREAKVQWKVDNALQSGNSQESVTEQDSKDSTYSLSSTLTLSKADYEKHKVYACEVTHQGLSSPVTKSFNRGEC

SEQ ID NO: 31 - protein, 123 aa, synthetic construct [sequence omitted]

SEQ ID NO: 32 - DNA, 369 bp, synthetic construct
  source 1..369: mol_type = other DNA; note = nucleic acid encoding HC of Bevacizumab
gaggtgcagctggtcgagtccgggggggggctggtgcagccaggcgggtctctgaggctgagttgcgccgcttcagggtacaccttcacaaactatggaatgaattgggtgcgccaggcaccaggaaagggactggagtgggtcggctggatcaacacttacaccggggaacctacctatgcagccgactttaagcggcggttcaccttcagcctggatacaagcaaatccactgcctacctgcagatgaacagcctgcgagctgaggacaccgcagtctactattgtgctaaatatccccactactatgggagcagccattggtattttgacgtgtgggggcaggggactctggtgacagtgagcagc

SEQ ID NO: 33 - protein, 107 aa, synthetic construct [sequence omitted]

SEQ ID NO: 34 - DNA, 321 bp, synthetic construct
  source 1..321: mol_type = other DNA; note = nucleic acid encoding LC of Bevacizumab
gatattcagatgactcagagcccctcctccctgtccgcctctgtgggcgacagggtcaccatcacatgcagtgcttcacaggatatttccaactacctgaattggtatcagcagaagccaggaaaagcacccaaggtgctgatctacttcactagctccctgcactcaggagtgccaagccggttcagcggatccggatctggaaccgactttactctgaccatttctagtctgcagcctgaggatttcgctacatactattgccagcagtattctaccgtgccatggacatttggccaggggactaaagtcgagatcaag

SEQ ID NO: 35 - protein, 108 aa, synthetic construct
  source 1..108: note = 14C12L1(M)V
DIQMTQSPSSMSASVGDRVTFTCRASQDINTYLSWFQQKPGKSPKTLIYRANRLVSGVPSRFSGSGSGQDYTLTISSLQPEDMATYYCLQYDEFPLTFGAGTKLELKR

SEQ ID NO: 36 - protein, 20 aa, synthetic construct
  source 1..20: note = linker
GGGGSGGGGSGGGGSGGGGS

SEQ ID NO: 37 - protein, 15 aa, synthetic construct
  source 1..15: note = linker
GGGGSGGGGSGGGGS

SEQ ID NO: 38 - protein, 453 aa, synthetic construct
  source 1..453: note = amino acid sequence of HC of immunoglobulin in VP101 (hG1WT)
EVQLVESGGGLVQPGGSLRLSCAASGYTFTNYGMNWVRQAPGKGLEWVGWINTYTGEPTYAADFKRRFTFSLDTSKSTAYLQMNSLRAEDTAVYYCAKYPHYYGSSHWYFDVWGQGTLVTVSSASTKGPSVFPLAPSSKSTSGGTAALGCLVKDYFPEPVTVSWNSGALTSGVHTFPAVLQSSGLYSLSSVVTVPSSSLGTQTYICNVNHKPSNTKVDKKVEPKSCDKTHTCPPCPAPELLGGPSVFLFPPKPKDTLMISRTPEVTCVVVDVSHEDPEVKFNWYVDGVEVHNAKTKPREEQYNSTYRVVSVLTVLHQDWLNGKEYKCKVSNKALPAPIEKTISKAKGQPREPQVYTLPPSRDELTKNQVSLTCLVKGFYPSDIAVEWESNGQPENNYKTTPPVLDSDGSFFLYSKLTVDKSRWQQGNVFSCSVMHEALHNHYTQKSLSLSPGK

SEQ ID NO: 39 - DNA, 1359 bp, synthetic construct
  source 1..1359: mol_type = other DNA; note = nucleic acid encoding HC of immunoglobulin in VP101 (hG1WT)
gaggtgcagctggtcgagtccgggggggggctggtgcagccaggcgggtctctgaggctgagttgcgccgcttcagggtacaccttcacaaactatggaatgaattgggtgcgccaggcaccaggaaagggactggagtgggtcggctggatcaacacttacaccggggaacctacctatgcagccgactttaagcggcggttcaccttcagcctggatacaagcaaatccactgcctacctgcagatgaacagcctgcgagctgaggacaccgcagtctactattgtgctaaatatccccactactatgggagcagccattggtattttgacgtgtgggggcaggggactctggtgacagtgagcagcgcaagcaccaaagggcccagcgtgtttcctctcgccccctcctccaaaagcaccagcggaggaaccgctgctctcggatgtctggtgaaggactacttccctgaacccgtcaccgtgagctggaatagcggcgctctgacaagcggagtccatacattccctgctgtgctgcaaagcagcggactctattccctgtccagcgtcgtcacagtgcccagcagcagcctgggcacccagacctacatctgtaacgtcaaccacaagccctccaacaccaaggtggacaagaaagtggagcccaaatcctgcgacaagacacacacctgtcccccctgtcctgctcccgaactcctcggaggccctagcgtcttcctctttcctcccaaacccaaggacaccctcatgatcagcagaacccctgaagtcacctgtgtcgtcgtggatgtcagccatgaggaccccgaggtgaaattcaactggtatgtcgatggcgtcgaggtgcacaacgccaaaaccaagcccagggaggaacagtacaactccacctacagggtggtgtccgtgctgacagtcctccaccaggactggctgaacggcaaggagtacaagtgcaaggtgtccaacaaggctctccctgcccccattgagaagaccatcagcaaggccaaaggccaacccagggagccccaggtctatacactgcctccctccagggacgaactcaccaagaaccaggtgtccctgacctgcctggtcaagggcttttatcccagcgacatcgccgtcgagtgggagtccaacggacagcccgagaataactacaagaccacccctcctgtcctcgactccgacggctccttcttcctgtacagcaaactgaccgtcgataaatctaggtggcagcagggcaacgtgttctcttgttccgtgatgcatgaagcactgcacaaccattatacccagaagtctctgagcctgtcccccggcaag

SEQ ID NO: 40 - protein, 450 aa, synthetic construct
  source 1..450: note = amino acid sequence of HC of immunoglobulin in VP101 (hG4WT)
EVQLVESGGGLVQPGGSLRLSCAASGYTFTNYGMNWVRQAPGKGLEWVGWINTYTGEPTYAADFKRRFTFSLDTSKSTAYLQMNSLRAEDTAVYYCAKYPHYYGSSHWYFDVWGQGTLVTVSSASTKGPSVFPLAPCSRSTSESTAALGCLVKDYFPEPVTVSWNSGALTSGVHTFPAVLQSSGLYSLSSVVTVPSSSLGTKTYTCNVDHKPSNTKVDKRVESKYGPPCPPCPAPEFLGGPSVFLFPPKPKDTLMISRTPEVTCVVVDVSQEDPEVQFNWYVDGVEVHNAKTKPREEQFNSTYRVVSVLTVLHQDWLNGKEYKCKVSNKGLPSSIEKTISKAKGQPREPQVYTLPPSQEEMTKNQVSLTCLVKGFYPSDIAVEWESNGQPENNYKTTPPVLDSDGSFFLYSRLTVDKSRWQEGNVFSCSVMHEALHNHYTQKSLSLSLGK

SEQ ID NO: 41 - DNA, 1350 bp, synthetic construct
  source 1..1350: mol_type = other DNA; note = nucleic acid encoding HC of immunoglobulin in VP101 (hG4WT)
gaggtgcagctggtcgagtccgggggggggctggtgcagccaggcgggtctctgaggctgagttgcgccgcttcagggtacaccttcacaaactatggaatgaattgggtgcgccaggcaccaggaaagggactggagtgggtcggctggatcaacacttacaccggggaacctacctatgcagccgactttaagcggcggttcaccttcagcctggatacaagcaaatccactgcctacctgcagatgaacagcctgcgagctgaggacaccgcagtctactattgtgctaaatatccccactactatgggagcagccattggtattttgacgtgtgggggcaggggactctggtgacagtgagcagcgcaagcaccaaagggccctcggtcttccccctggcgccctgctccaggagcacctccgagagcacagccgccctgggctgcctggtcaaggactacttccccgaaccggtgacggtgtcgtggaactcaggcgccctgaccagcggcgtgcacaccttcccggctgtcctacagtcctcaggactctactccctcagcagcgtggtgaccgtgccctccagcagcttgggcacgaagacctacacctgcaacgtagatcacaagcccagcaacaccaaggtggacaagagagttgagtccaaatatggtcccccatgcccaccatgcccagcacctgagttcctggggggaccatcagtcttcctgttccccccaaaacccaaggacactctcatgatctcccggacccctgaggtcacgtgcgtggtggtggacgtgagccaggaagaccccgaggtccagttcaactggtacgtggatggcgtggaggtgcataatgccaagacaaagccgcgggaggagcagttcaacagcacgtaccgtgtggtcagcgtcctcaccgtcctgcaccaggactggctgaacggcaaggagtacaagtgcaaggtctccaacaaaggcctcccgtcctccatcgagaaaaccatctccaaagccaaagggcagccccgagagccacaggtgtacaccctgcccccatcccaggaggagatgaccaagaaccaggtcagcctgacctgcctggtcaaaggcttctaccccagcgacatcgccgtggagtgggagagcaatgggcagccggagaacaactacaagaccacgcctcccgtgctggactccgacggctccttcttcctctacagcaggctaaccgtggacaagagcaggtggcaggaggggaatgtcttctcatgctccgtgatgcatgaggctctgcacaaccactacacacagaagtctctgagcctgtccctcggcaag

SEQ ID NO: 42 - protein, 453 aa, synthetic construct
  source 1..453: note = amino acid sequence of HC of immunoglobulin in VP101(hG1DM)
EVQLVESGGGLVQPGGSLRLSCAASGYTFTNYGMNWVRQAPGKGLEWVGWINTYTGEPTYAADFKRRFTFSLDTSKSTAYLQMNSLRAEDTAVYYCAKYPHYYGSSHWYFDVWGQGTLVTVSSASTKGPSVFPLAPSSKSTSGGTAALGCLVKDYFPEPVTVSWNSGALTSGVHTFPAVLQSSGLYSLSSVVTVPSSSLGTQTYICNVNHKPSNTKVDKKVEPKSCDKTHTCPPCPAPEAAGGPSVFLFPPKPKDTLMISRTPEVTCVVVDVSHEDPEVKFNWYVDGVEVHNAKTKPREEQYNSTYRVVSVLTVLHQDWLNGKEYKCKVSNKALPAPIEKTISKAKGQPREPQVYTLPPSRDELTKNQVSLTCLVKGFYPSDIAVEWESNGQPENNYKTTPPVLDSDGSFFLYSKLTVDKSRWQQGNVFSCSVMHEALHNHYTQKSLSLSPGK

SEQ ID NO: 43 - DNA, 1359 bp, synthetic construct
  source 1..1359: mol_type = other DNA; note = nucleic acid encoding HC of immunoglobulin in VP101(hG1DM)
gaggtgcagctggtcgagtccgggggggggctggtgcagccaggcgggtctctgaggctgagttgcgccgcttcagggtacaccttcacaaactatggaatgaattgggtgcgccaggcaccaggaaagggactggagtgggtcggctggatcaacacttacaccggggaacctacctatgcagccgactttaagcggcggttcaccttcagcctggatacaagcaaatccactgcctacctgcagatgaacagcctgcgagctgaggacaccgcagtctactattgtgctaaatatccccactactatgggagcagccattggtattttgacgtgtgggggcaggggactctggtgacagtgagcagcgcaagcaccaaagggcccagcgtgtttcctctcgccccctcctccaaaagcaccagcggaggaaccgctgctctcggatgtctggtgaaggactacttccctgaacccgtcaccgtgagctggaatagcggcgctctgacaagcggagtccatacattccctgctgtgctgcaaagcagcggactctattccctgtccagcgtcgtcacagtgcccagcagcagcctgggcacccagacctacatctgtaacgtcaaccacaagccctccaacaccaaggtggacaagaaagtggagcccaaatcctgcgacaagacacacacctgtcccccctgtcctgctcccgaagctgctggaggccctagcgtcttcctctttcctcccaaacccaaggacaccctcatgatcagcagaacccctgaagtcacctgtgtcgtcgtggatgtcagccatgaggaccccgaggtgaaattcaactggtatgtcgatggcgtcgaggtgcacaacgccaaaaccaagcccagggaggaacagtacaactccacctacagggtggtgtccgtgctgacagtcctccaccaggactggctgaacggcaaggagtacaagtgcaaggtgtccaacaaggctctccctgcccccattgagaagaccatcagcaaggccaaaggccaacccagggagccccaggtctatacactgcctccctccagggacgaactcaccaagaaccaggtgtccctgacctgcctggtcaagggcttttatcccagcgacatcgccgtcgagtgggagtccaacggacagcccgagaataactacaagaccacccctcctgtcctcgactccgacggctccttcttcctgtacagcaaactgaccgtcgataaatctaggtggcagcagggcaacgtgttctcttgttccgtgatgcatgaagcactgcacaaccattatacccagaagtctctgagcctgtcccccggcaag

SEQ ID NO: 44 - protein, 214 aa, synthetic construct
  source 1..214: note = amino acid sequence of LC of immunoglobulin in VP101(hG1DM)
DIQMTQSPSSLSASVGDRVTITCSASQDISNYLNWYQQKPGKAPKVLIYFTSSLHSGVPSRFSGSGSGTDFTLTISSLQPEDFATYYCQQYSTVPWTFGQGTKVEIKRTVAAPSVFIFPPSDEQLKSGTASVVCLLNNFYPREAKVQWKVDNALQSGNSQESVTEQDSKDSTYSLSSTLTLSKADYEKHKVYACEVTHQGLSSPVTKSFNRGEC

SEQ ID NO: 45 - DNA, 642 bp, synthetic construct
  source 1..642: mol_type = other DNA; note = nucleic acid encoding LC of immunoglobulin in VP101(hG1DM)
gatattcagatgactcagagcccctcctccctgtccgcctctgtgggcgacagggtcaccatcacatgcagtgcttcacaggatatttccaactacctgaattggtatcagcagaagccaggaaaagcacccaaggtgctgatctacttcactagctccctgcactcaggagtgccaagccggttcagcggatccggatctggaaccgactttactctgaccatttctagtctgcagcctgaggatttcgctacatactattgccagcagtattctaccgtgccatggacatttggccaggggactaaagtcgagatcaagcggaccgtggccgctcccagtgtcttcatttttccccctagcgacgaacagctgaaatccgggacagcctctgtggtctgtctgctgaacaacttctaccctagagaggcaaaagtgcagtggaaggtcgataacgccctgcagagtggcaattcacaggagagcgtgacagaacaggactccaaagattctacttatagtctgtcaagcacactgactctgagcaaggctgactacgaaaagcataaagtgtatgcatgtgaggtcacccaccaggggctgagcagtccagtcaccaagtcattcaacagaggcgagtgc

SEQ ID NO: 46 - protein, 121 aa, synthetic construct
  source 1..121: note = amino acid sequence of 26B12VH
EVQLQESGPGLVKPSQSLSLTCTVTGHSFTSDYAWNWIRQFPGNRLEWMGYISYSDSTNYNPSLKSRISITRDTSKNQFFLQMNSVTTEDTATYYCARLDYGNYGGAMDYWGQGTSVTVSS

SEQ ID NO: 47 - DNA, 363 bp, synthetic construct
  source 1..363: mol_type = other DNA; note = nucleic acid sequence of 26B12VH
gaggtgcagctgcaggagtctggacctggcctggtgaaaccctctcagtctctgtccctcacctgcactgtcactggccactcattcaccagtgattatgcctggaactggatccggcagtttccaggaaacagactggagtggatgggctacataagctacagtgatagcactaactacaacccatctctcaaaagtcgaatctctatcactcgagacacatccaagaaccagttcttcttgcagatgaattctgtgactactgaggacacagccacatattactgtgcaagattggactatggtaactacggtggggctatggactactggggtcaagggacctcagtcaccgtctcctca

SEQ ID NO: 48 - protein, 107 aa, synthetic construct
  source 1..107: note = amino acid sequence of 26B12VL
DIVLTQSHEFMSTSLRDRVSITCKSSQHVSTAVAWYQQKPGQSPKLLIYSASYRYTGVPDRFTGSGSGTDFTFTISSVKAEDLAVYYCQQHYITPWTFGGGTKLEIK

SEQ ID NO: 49 - DNA, 321 bp, synthetic construct
  source 1..321: mol_type = other DNA; note = nucleic acid sequence of 26B12VL
gatattgtgctaactcagtctcacgaattcatgtccacctcattacgagacagggtcagcatcacctgcaaatccagtcaacatgtgagtactgctgtagcctggtatcaacagaaaccaggacaatctcctaaactactgatttactcggcatcctaccggtacactggagtccctgatcgcttcactggcagtggatctgggacggatttcactttcaccatcagcagtgtgaaggctgaagacctggcagtttattactgtcagcaacattatattactccgtggacgttcggtggaggcaccaagctggaaataaaa

SEQ ID NO: 50 - protein, 121 aa, synthetic construct
  source 1..121: note = amino acid sequence of 26B12H1VH
DVQLQESGPGLVKPSQTLSLTCTVSGHSFTSDYAWNWIRQFPGKGLEWIGYISYSDSTNYNPSLKSRITISRDTSKNQFFLQLNSVTAADTATYYCARLDYGNYGGAMDYWGQGTSVTVSS

SEQ ID NO: 51 - DNA, 363 bp, synthetic construct
  source 1..363: mol_type = other DNA; note = nucleic acid sequence of 26B12H1VH
gatgtgcagctgcaggagagcggccccggactggtgaagccttcccagaccctgtctctgacctgtacagtgtctggccacagcttcacatccgactacgcctggaactggatcaggcagtttccaggcaagggcctggagtggatcggctacatctcttatagcgactccaccaactataatccctctctgaagagccggatcaccatcagcagagatacatccaagaaccagttctttctgcagctgaacagcgtgacagccgccgacaccgccacatactattgcgcccggctggactacggcaattatggcggagccatggattactggggccagggcacctccgtgacagtgagctcc

SEQ ID NO: 52 - protein, 121 aa, synthetic construct
  source 1..121: note = amino acid sequence of 26B12H2VH
DVQLQESGPGLVKPSQTLSLTCTVSGHSFTSDYAWSWIRQPPGKGLEWIGYISYSDSTNYNPSLKSRVTISRDTSKNQFSLKLSSVTAADTAVYYCARLDYGNYGGAMDYWGQGTSVTVSS

SEQ ID NO: 53 - DNA, 363 bp, synthetic construct
  source 1..363: mol_type = other DNA; note = nucleic acid sequence of 26B12H2VH
gatgtgcagctgcaggagtctggcccaggactggtgaagccaagccagaccctgtccctgacctgtacagtgtccggccactcttttacaagcgactacgcctggtcttggatcaggcagccccctggcaagggactggagtggatcggctacatctcctattctgacagcaccaactataatccctccctgaagtctcgggtgaccatctctagagatacaagcaagaaccagttctccctgaagctgagctccgtgaccgcagcagacacagccgtgtactattgcgcccggctggactacggcaattatggcggagccatggattactggggccagggcaccagcgtgacagtgtctagc

SEQ ID NO: 54 - protein, 121 aa, synthetic construct
  source 1..121: note = amino acid sequence of 26B12H3VH
DVQLQESGPGLVKPSQTLSLTCTVSGHSFTSDYAWSWIRQPPGKGLEWIGYISYSDSTNYNPSLKSRVTISVDTSKNQFSLKLSSVTAADTAVYYCARLDYGNYGGAMDYWGQGTSVTVSS

SEQ ID NO: 55 - DNA, 363 bp, synthetic construct
  source 1..363: mol_type = other DNA; note = nucleic acid sequence of 26B12H3VH
gatgtgcagctgcaggagtctggcccaggactggtgaagccaagccagaccctgtccctgacctgtacagtgtccggccactcttttacaagcgactacgcctggtcttggatcagacagccccctggcaagggactggagtggatcggctacatctcctattctgacagcaccaactataatccctccctgaagtctagagtgaccatctctgtggatacaagcaagaaccagttctccctgaagctgagctccgtgaccgcagcagacacagccgtgtactattgcgcccggctggactacggcaattatggcggagccatggattactggggccagggcaccagcgtgacagtgtctagc

SEQ ID NO: 56 - protein, 121 aa, synthetic construct
  source 1..121: note = amino acid sequence of 26B12H4VH
DVQLQESGPGLVKPSQTLSLTCTVSGHSFTSDYAWNWIRQFPGKGLEWMGYISYSDSTNYNPSLKSRITISRDTSKNQFFLQLNSVTAADTATYYCARLDYGNYGGAMDYWGQGTSVTVSS

SEQ ID NO: 57 - DNA, 363 bp, synthetic construct
  source 1..363: mol_type = other DNA; note = nucleic acid sequence of 26B12H4VH
gatgtgcagctgcaggagagcggccccggactggtgaagccttcccagaccctgtctctgacctgtacagtgtctggccacagcttcacatccgactacgcctggaactggatcaggcagtttccaggcaagggcctggagtggatgggctacatctcttatagcgactccaccaactataatccctctctgaagagccggatcaccatcagcagagatacatccaagaaccagttctttctgcagctgaacagcgtgacagccgccgacaccgccacatactattgcgcccggctggactacggcaattatggcggagccatggattactggggccagggcacctccgtgacagtgagctcc

SEQ ID NO: 58 - protein, 107 aa, synthetic construct
  source 1..107: note = amino acid sequence of 26B12L1VL
DIQMTQSPKSLSTSVGDRVTITCRSSQHVSTAVAWYQQKPGKSPKLLIYSASYRYSGVPDRFSGSGSGTDFTFTISSVQPEDFATYYCQQHYITPWTFGGGTKLEIK

SEQ ID NO: 59 - DNA, 321 bp, synthetic construct
  source 1..321: mol_type = other DNA; note = nucleic acid sequence of 26B12L1VL
gacatccagatgacccagtcccctaagtccctgtctacaagcgtgggcgatcgggtgaccatcacatgtagaagctcccagcacgtgtctaccgcagtggcatggtaccagcagaagccaggcaagagccctaagctgctgatctattccgcctcttacaggtattccggagtgccagaccggtttagcggctccggctctggcaccgatttcacctttacaatctctagcgtgcagccagaggacttcgccacatactattgccagcagcactacatcaccccatggaccttcggcggcggcacaaagctggagatcaag

SEQ ID NO: 60 - protein, 107 aa, synthetic construct
  source 1..107: note = amino acid sequence of 26B12L2VL
DIQMTQSPSSLSASVGDRVTITCRSSQHVSTALAWYQQKPGKSPKLLIYSASSRYSGVPDRFSGSGSGTDFTFTISSLQPEDFATYYCQQHYITPWTFGGGTKLEIK

SEQ ID NO: 61 - DNA, 321 bp, synthetic construct
  source 1..321: mol_type = other DNA; note = nucleic acid sequence of 26B12L2VL
gacatccagatgacccagtcccctagctccctgtctgccagcgtgggcgatagggtgaccatcacatgtagatctagccagcacgtgtctacagccctggcatggtaccagcagaagccaggcaagagccctaagctgctgatctactccgcctcctctaggtattctggagtgccagaccggttttccggctctggcagcggcaccgatttcacctttacaatcagctccctgcagccagaggacttcgccacatactattgccagcagcactatatcaccccatggaccttcggcggcggcaccaagctggagatcaag

SEQ ID NO: 62 - protein, 107 aa, synthetic construct
  source 1..107: note = amino acid sequence of 26B12L3VL
DIQMTQSPSSLSASVGDRVTITCRASQHVSTALAWYQQKPGKAPKLLIYSASSLQSGVPSRFSGSGSGTDFTLTISSLQPEDFATYYCQQHYITPWTFGGGTKLEIK

SEQ ID NO: 63 - DNA, 321 bp, synthetic construct
  source 1..321: mol_type = other DNA; note = nucleic acid sequence of 26B12L3VL
gacatccagatgacccagtcccctagctccctgagcgcctccgtgggcgatagggtgaccatcacatgtagagcctctcagcacgtgagcacagccctggcatggtaccagcagaagccaggcaaggcccctaagctgctgatctatagcgcctctagcctgcagtccggagtgccatctcggttctctggcagcggctccggaaccgactttaccctgacaatctcctctctgcagccagaggatttcgccacatactattgccagcagcactacatcaccccatggaccttcggcggcggcaccaagctggagatcaag

SEQ ID NO: 64 - protein, 107 aa, synthetic construct
  source 1..107: note = amino acid sequence of 26B12L4VL
DIQMTQSPKSMSTSVGDRVTITCRSSQHVSTAVAWYQQKPGKSPKLLIYSASYRYSGVPDRFSGSGSGTDFTFTISSVQPEDFATYYCQQHYITPWTFGGGTKLEIK

SEQ ID NO: 65 - DNA, 321 bp, synthetic construct
  source 1..321: mol_type = other DNA; note = nucleic acid sequence of 26B12L4VL
gacatccagatgacccagtcccctaagtccatgtctacaagcgtgggcgacagggtgaccatcacatgtagaagctcccagcacgtgtctaccgcagtggcatggtaccagcagaagccaggcaagagccctaagctgctgatctattccgcctcttacaggtattccggagtgccagaccggtttagcggctccggctctggcaccgatttcacctttacaatctctagcgtgcagccagaggacttcgccacatactattgccagcagcactacatcaccccatggaccttcggcggcggcacaaagctggagatcaag

SEQ ID NO: 66 - protein, 447 aa, synthetic construct
  source 1..447: note = amino acid sequence of HC of 26B12H2L2(hG4DM)
DVQLQESGPGLVKPSQTLSLTCTVSGHSFTSDYAWSWIRQPPGKGLEWIGYISYSDSTNYNPSLKSRVTISRDTSKNQFSLKLSSVTAADTAVYYCARLDYGNYGGAMDYWGQGTSVTVSSASTKGPSVFPLAPCSRSTSESTAALGCLVKDYFPEPVTVSWNSGALTSGVHTFPAVLQSSGLYSLSSVVTVPSSSLGTKTYTCNVDHKPSNTKVDKRVESKYGPPCPPCPAPEAAGGPSVFLFPPKPKDTLMISRTPEVTCVVVDVSQEDPEVQFNWYVDGVEVHNAKTKPREEQFNSTYRVVSVLTVLHQDWLNGKEYKCKVSNKGLPSSIEKTISKAKGQPREPQVYTLPPSQEEMTKNQVSLTCLVKGFYPSDIAVEWESNGQPENNYKTTPPVLDSDGSFFLYSRLTVDKSRWQEGNVFSCSVMHEALHNHYTQKSLSLSLG

SEQ ID NO: 67 - DNA, 1341 bp, synthetic construct
  source 1..1341: mol_type = other DNA; note = nucleic acid encoding HC of 26B12H2L2(hG4DM)
gatgtgcagctgcaggagtctggcccaggactggtgaagccaagccagaccctgtccctgacctgtacagtgtccggccactcttttacaagcgactacgcctggtcttggatcaggcagccccctggcaagggactggagtggatcggctacatctcctattctgacagcaccaactataatccctccctgaagtctcgggtgaccatctctagagatacaagcaagaaccagttctccctgaagctgagctccgtgaccgcagcagacacagccgtgtactattgcgcccggctggactacggcaattatggcggagccatggattactggggccagggcaccagcgtgacagtgtctagcgcctccacaaaggggccctcggtcttccccctggcgccctgctccaggagcacctccgagagcacagccgccctgggctgcctggtcaaggactacttccccgaaccggtgacggtgtcgtggaactcaggcgccctgaccagcggcgtacacaccttcccggctgtcctacagtcctcaggactctactccctcagcagcgtggtgaccgtgccctccagcagcttgggcacgaagacctacacctgcaacgtagatcacaagcccagcaacaccaaggtggacaagagagttgagtccaaatatggtcccccatgcccaccatgcccagcacctgaggccgctgggggaccatcagtcttcctgttccccccaaaacccaaggacactctcatgatctcccggacccctgaggtcacgtgcgtggtggtggacgtgagccaggaagaccccgaggtccagttcaactggtacgtggatggcgtggaggtgcataatgccaagacaaagccgcgggaggagcagttcaacagcacgtaccgtgtggtcagcgtcctcaccgtcctgcaccaggactggctgaacggcaaggagtacaagtgcaaggtctccaacaaaggcctcccgtcctccatcgagaaaaccatctccaaagccaaagggcagccccgagagccacaggtgtacaccctgcccccatcccaggaggagatgaccaagaaccaggtcagcctgacctgcctggtcaaaggcttctaccccagcgacatcgccgtggagtgggagagcaatgggcagccggagaacaactacaagaccacgcctcccgtgctggactccgacggctccttcttcctctacagcaggctaaccgtggacaagagcaggtggcaggaggggaatgtcttctcatgctccgtgatgcatgaggctctgcacaaccactacacacagaagagcctctccctgtctctgggt

SEQ ID NO: 68 - protein, 214 aa, synthetic construct
  source 1..214: note = amino acid sequence of LC of 26B12H2L2(hG4DM)
DIQMTQSPSSLSASVGDRVTITCRSSQHVSTALAWYQQKPGKSPKLLIYSASSRYSGVPDRFSGSGSGTDFTFTISSLQPEDFATYYCQQHYITPWTFGGGTKLEIKRTVAAPSVFIFPPSDEQLKSGTASVVCLLNNFYPREAKVQWKVDNALQSGNSQESVTEQDSKDSTYSLSSTLTLSKADYEKHKVYACEVTHQGLSSPVTKSFNRGEC

SEQ ID NO: 69 - DNA, 642 bp, synthetic construct
  source 1..642: mol_type = other DNA; note = nucleic acid encoding LC of 26B12H2L2(hG4DM)
gacatccagatgacccagtcccctagctccctgtctgccagcgtgggcgatagggtgaccatcacatgtagatctagccagcacgtgtctacagccctggcatggtaccagcagaagccaggcaagagccctaagctgctgatctactccgcctcctctaggtattctggagtgccagaccggttttccggctctggcagcggcaccgatttcacctttacaatcagctccctgcagccagaggacttcgccacatactattgccagcagcactatatcaccccatggaccttcggcggcggcaccaagctggagatcaagcgtacggtggcagccccatctgtcttcatttttccccctagtgacgagcagctgaaatccggaacagcctctgtggtctgtctgctgaacaatttctaccctcgcgaagccaaggtgcagtggaaagtcgataacgctctgcagagtggcaattcacaggagagcgtgactgaacaggactccaaggattctacctatagtctgagctccactctgaccctgtccaaagcagattacgaaaagcacaaagtgtatgcctgtgaggtcacccaccaggggctgagttctccagtcaccaaatccttcaacagaggcgaatgt

SEQ ID NO: 70 - protein, 451 aa, synthetic construct
  source 1..451: note = amino acid sequence of HC of 26B12H2L2(hG1DM)
DVQLQESGPGLVKPSQTLSLTCTVSGHSFTSDYAWSWIRQPPGKGLEWIGYISYSDSTNYNPSLKSRVTISRDTSKNQFSLKLSSVTAADTAVYYCARLDYGNYGGAMDYWGQGTSVTVSSASTKGPSVFPLAPSSKSTSGGTAALGCLVKDYFPEPVTVSWNSGALTSGVHTFPAVLQSSGLYSLSSVVTVPSSSLGTQTYICNVNHKPSNTKVDKKVEPKSCDKTHTCPPCPAPEAAGGPSVFLFPPKPKDTLMISRTPEVTCVVVDVSHEDPEVKFNWYVDGVEVHNAKTKPREEQYNSTYRVVSVLTVLHQDWLNGKEYKCKVSNKALPAPIEKTISKAKGQPREPQVYTLPPSRDELTKNQVSLTCLVKGFYPSDIAVEWESNGQPENNYKTTPPVLDSDGSFFLYSKLTVDKSRWQQGNVFSCSVMHEALHNHYTQKSLSLSPGK

SEQ ID NO: 71 - DNA, 1353 bp, synthetic construct
  source 1..1353: mol_type = other DNA; note = nucleic acid encoding HC of 26B12H2L2(hG1DM)
gatgtgcagctgcaggagtctggcccaggactggtgaagccaagccagaccctgtccctgacctgtacagtgtccggccactcttttacaagcgactacgcctggtcttggatcaggcagccccctggcaagggactggagtggatcggctacatctcctattctgacagcaccaactataatccctccctgaagtctcgggtgaccatctctagagatacaagcaagaaccagttctccctgaagctgagctccgtgaccgcagcagacacagccgtgtactattgcgcccggctggactacggcaattatggcggagccatggattactggggccagggcaccagcgtgacagtgtctagcgcctctaccaaggggcccagcgtgtttcctctcgccccctcctccaaaagcaccagcggaggaaccgctgctctcggatgtctggtgaaggactacttccctgaacccgtcaccgtgagctggaatagcggcgctctgacaagcggagtccatacattccctgctgtgctgcaaagcagcggactctattccctgtccagcgtcgtcacagtgcccagcagcagcctgggcacccagacctacatctgtaacgtcaaccacaagccctccaacaccaaggtggacaagaaagtggagcccaaatcctgcgacaagacacacacctgtcccccctgtcctgctcccgaagctgctggaggccctagcgtcttcctctttcctcccaaacccaaggacaccctcatgatcagcagaacccctgaagtcacctgtgtcgtcgtggatgtcagccatgaggaccccgaggtgaaattcaactggtatgtcgatggcgtcgaggtgcacaacgccaaaaccaagcccagggaggaacagtacaactccacctacagggtggtgtccgtgctgacagtcctccaccaggactggctgaacggcaaggagtacaagtgcaaggtgtccaacaaggctctccctgcccccattgagaagaccatcagcaaggccaaaggccaacccagggagccccaggtctatacactgcctccctccagggacgaactcaccaagaaccaggtgtccctgacctgcctggtcaagggcttttatcccagcgacatcgccgtcgagtgggagtccaacggacagcccgagaataactacaagaccacccctcctgtcctcgactccgacggctccttcttcctgtacagcaagctgaccgtggacaaaagcaggtggcagcagggaaacgtgttctcctgcagcgtgatgcacgaagccctccacaaccactacacccagaaaagcctgtccctgagccccggcaaa

SEQ ID NO: 72 - protein, 136 aa, synthetic construct
  source 1..136: note = extracellular domain fragment of TGF-betaRII
IPPHVQKSVNNDMIVTDNNGAVKFPQLCKFCDVRFSTCDNQKSCMSNCSITSICEKPQEVCVAVWRKNDENITLETVCHDPKLPYHDFILEDAASPKCIMKEKKKPGETFFMCSCSSDECNDNIIFSEEYNTSNPD

SEQ ID NO: 73 - protein, 503 aa, synthetic construct
  source 1..503: note = TGF-betaRI
MEAAVAAPRPRLLLLVLAAAAAAAAALLPGATALQCFCHLCTKDNFTCVTDGLCFVSVTETTDKVIHNSMCIAEIDLIPRDRPFVCAPSSKTGSVTTTYCCNQDHCNKIELPTTVKSSPGLGPVELAAVIAGPVCFVCISLMLMVYICHNRTVIHHRVPNEEDPSLDRPFISEGTTLKDLIYDMTTSGSGSGLPLLVQRTIARTIVLQESIGKGRFGEVWRGKWRGEEVAVKIFSSREERSWFREAEIYQTVMLRHENILGFIAADNKDNGTWTQLWLVSDYHEHGSLFDYLNRYTVTVEGMIKLALSTASGLAHLHMEIVGTQGKPAIAHRDLKSKNILVKKNGTCCIADLGLAVRHDSATDTIDIAPNHRVGTKRYMAPEVLDDSINMKHFESFKRADIYAMGLVFWEIARRCSIGGIHEDYQLPYYDLVPSDPSVEEMRKVVCEQKLRPNIPNRWQSCEALRVMAKIMRECWYANGAARLTALRIKKTLSQLSQQEGIKM

SEQ ID NO: 74 - protein, 93 aa, synthetic construct
  source 1..93: note = extracellular domain of TGF-betaRI
LQCFCHLCTKDNFTCVTDGLCFVSVTETTDKVIHNSMCIAEIDLIPRDRPFVCAPSSKTGSVTTTYCCNQDHCNKIELPTTVKSSPGLGPVEL

SEQ ID NO: 75 - protein, 567 aa, synthetic construct
  source 1..567: note = TGF-betaRII
MGRGLLRGLWPLHIVLWTRIASTIPPHVQKSVNNDMIVTDNNGAVKFPQLCKFCDVRFSTCDNQKSCMSNCSITSICEKPQEVCVAVWRKNDENITLETVCHDPKLPYHDFILEDAASPKCIMKEKKKPGETFFMCSCSSDECNDNIIFSEEYNTSNPDLLLVIFQVTGISLLPPLGVAISVIIIFYCYRVNRQQKLSSTWETGKTRKLMEFSEHCAIILEDDRSDISSTCANNINHNTELLPIELDTLVGKGRFAEVYKAKLKQNTSEQFETVAVKIFPYEEYASWKTEKDIFSDINLKHENILQFLTAEERKTELGKQYWLITAFHAKGNLQEYLTRHVISWEDLRKLGSSLARGIAHLHSDHTPCGRPKMPIVHRDLKSSNILVKNDLTCCLCDFGLSLRLDPTLSVDDLANSGQVGTARYMAPEVLESRMNLENVESFKQTDVYSMALVLWEMTSRCNAVGEVKDYEPPFGSKVREHPCVESMKDNVLRDRGRPEIPSFWLNHQGIQMVCETLTECWDHDPEARLTAQCVAERFSELEHLDRLSGRSCSEEKIPEDGSLNTTK

SEQ ID NO: 76 - protein, 144 aa, synthetic construct
  source 1..144: note = extracellular domain of TGF-betaRII
TIPPHVQKSVNNDMIVTDNNGAVKFPQLCKFCDVRFSTCDNQKSCMSNCSITSICEKPQEVCVAVWRKNDENITLETVCHDPKLPYHDFILEDAASPKCIMKEKKKPGETFFMCSCSSDECNDNIIFSEEYNTSNPDLLLVIFQ

SEQ ID NO: 77 - protein, 851 aa, synthetic construct
  source 1..851: note = TGF-betaRIII
MTSHYVIAIFALMSSCLATAGPEPGALCELSPVSASHPVQALMESFTVLSGCASRGTTGLPQEVHVLNLRTAGQGPGQLQREVTLHLNPISSVHIHHKSVVFLLNSPHPLVWHLKTERLATGVSRLFLVSEGSVVQFSSANFSLTAETEERNFPHGNEHLLNWARKEYGAVTSFTELKIARNIYIKVGEDQVFPPKCNIGKNFLSLNYLAEYLQPKAAEGCVMSSQPQNEEVHIIELITPNSNPYSAFQVDITIDIRPSQEDLEVVKNLILILKCKKSVNWVIKSFDVKGSLKIIAPNSIGFGKESERSMTMTKSIRDDIPSTQGNLVKWALDNGYSPITSYTMAPVANRFHLRLENNAEEMGDEEVHTIPPELRILLDPGALPALQNPPIRGGEGQNGGLPFPFPDISRRVWNEEGEDGLPRPKDPVIPSIQLFPGLREPEEVQGSVDIALSVKCDNEKMIVAVEKDSFQASGYSGMDVTLLDPTCKAKMNGTHFVLESPLNGCGTRPRWSALDGVVYYNSIVIQVPALGDSSGWPDGYEDLESGDNGFPGDMDEGDASLFTRPEIVVFNCSLQQVRNPSSFQEQPHGNITFNMELYNTDLFLVPSQGVFSVPENGHVYVEVSVTKAEQELGFAIQTCFISPYSNPDRMSHYTIIENICPKDESVKFYSPKRVHFPIPQADMDKKRFSFVFKPVFNTSLLFLQCELTLCTKMEKHPQKLPKCVPPDEACTSLDASIIWAMMQNKKTFTKPLAVIHHEAESKEKGPSMKEPNPISPPIFHGLDTLTVMGIAFAAFVIGALLTGALWYIYSHTGETAGRQQVPTSPPASENSSAAHSIGSTQSTPCSSSSTA

SEQ ID NO: 78 - protein, 767 aa, synthetic construct
  source 1..767: note = extracellular domain of TGF-betaRIII
GPEPGALCELSPVSASHPVQALMESFTVLSGCASRGTTGLPQEVHVLNLRTAGQGPGQLQREVTLHLNPISSVHIHHKSVVFLLNSPHPLVWHLKTERLATGVSRLFLVSEGSVVQFSSANFSLTAETEERNFPHGNEHLLNWARKEYGAVTSFTELKIARNIYIKVGEDQVFPPKCNIGKNFLSLNYLAEYLQPKAAEGCVMSSQPQNEEVHIIELITPNSNPYSAFQVDITIDIRPSQEDLEVVKNLILILKCKKSVNWVIKSFDVKGSLKIIAPNSIGFGKESERSMTMTKSIRDDIPSTQGNLVKWALDNGYSPITSYTMAPVANRFHLRLENNAEEMGDEEVHTIPPELRILLDPGALPALQNPPIRGGEGQNGGLPFPFPDISRRVWNEEGEDGLPRPKDPVIPSIQLFPGLREPEEVQGSVDIALSVKCDNEKMIVAVEKDSFQASGYSGMDVTLLDPTCKAKMNGTHFVLESPLNGCGTRPRWSALDGVVYYNSIVIQVPALGDSSGWPDGYEDLESGDNGFPGDMDEGDASLFTRPEIVVFNCSLQQVRNPSSFQEQPHGNITFNMELYNTDLFLVPSQGVFSVPENGHVYVEVSVTKAEQELGFAIQTCFISPYSNPDRMSHYTIIENICPKDESVKFYSPKRVHFPIPQADMDKKRFSFVFKPVFNTSLLFLQCELTLCTKMEKHPQKLPKCVPPDEACTSLDASIIWAMMQNKKTFTKPLAVIHHEAESKEKGPSMKEPNPISPPIFHGLDTLTV

SEQ ID NO: 79 - protein, 456 aa, synthetic construct
  source 1..456: note = Tiragolumab HC
EVQLQQSGPGLVKPSQTLSLTCAISGDSVSSNSAAWNWIRQSPSRGLEWLGKTYYRFKWYSDYAVSVKGRITINPDTSKNQFSLQLNSVTPEDTAVFYCTRESTTYDLLAGPFDYWGQGTLVTVSSASTKGPSVFPLAPSSKSTSGGTAALGCLVKDYFPEPVTVSWNSGALTSGVHTFPAVLQSSGLYSLSSVVTVPSSSLGTQTYICNVNHKPSNTKVDKKVEPKSCDKTHTCPPCPAPELLGGPSVFLFPPKPKDTLMISRTPEVTCVVVDVSHEDPEVKFNWYVDGVEVHNAKTKPREEQYNSTYRVVSVLTVLHQDWLNGKEYKCKVSNKALPAPIEKTISKAKGQPREPQVYTLPPSREEMTKNQVSLTCLVKGFYPSDIAVEWESNGQPENNYKTTPPVLDSDGSFFLYSKLTVDKSRWQQGNVFSCSVMHEALHNHYTQKSLSLSPGK

SEQ ID NO: 80 - protein, 220 aa, synthetic construct
  source 1..220: note = Tiragolumab LC
DIVMTQSPDSLAVSLGERATINCKSSQTVLYSSNNKKYLAWYQQKPGQPPNLLIYWASTRESGVPDRFSGSGSGTDFTLTISSLQAEDVAVYYCQQYYSTPFTFGPGTKVEIKRTVAAPSVFIFPPSDEQLKSGTASVVCLLNNFYPREAKVQWKVDNALQSGNSQESVTEQDSKDSTYSLSSTLTLSKADYEKHKVYACEVTHQGLSSPVTKSFNRGEC

SEQ ID NO: 81 - protein, 126 aa, synthetic construct
  source 1..126: note = RG6058(hG4) VH
EVQLQQSGPGLVKPSQTLSLTCAISGDSVSSNSAAWNWIRQSPSRGLEWLGKTYYRFKWYSDYAVSVKGRITINPDTSKNQFSLQLNSVTPEDTAVFYCTRESTTYDLLAGPFDYWGQGTLVTVSS

SEQ ID NO: 82 - protein, 113 aa, synthetic construct
  source 1..113: note = RG6058(hG4) VL
DIVMTQSPDSLAVSLGERATINCKSSQTVLYSSNNKKYLAWYQQKPGQPPNLLIYWASTRESGVPDRFSGSGSGTDFTLTISSLQAEDVAVYYCQQYYSTPFTFGPGTKVEIK

SEQ ID NO: 83 - protein, 21 aa, synthetic construct
  source 1..21: note = linker
GGGGSGGGGSGGGGSGGGGSG

SEQ ID NO: 84 - protein, 599 aa, synthetic construct
  source 1..599: note = HC of anti-HEL and anti-TGFbeta antibody
EVQLEQSGAELMKPGASVKISCKATGYTFTTYWIEWIKQRPGHSLEWIGEILPGSDSTYYNEKVKGKVTFTADASSNTAYMQLSSLTSEDSAVYYCARGDGFYVYWGQGTTLTVSSASTKGPSVFPLAPCSRSTSESTAALGCLVKDYFPEPVTVSWNSGALTSGVHTFPAVLQSSGLYSLSSVVTVPSSSLGTKTYTCNVDHKPSNTKVDKRVESKYGPPCPPCPAPEAAGGPSVFLFPPKPKDTLMISRTPEVTCVVVDVSQEDPEVQFNWYVDGVEVHNAKTKPREEQFNSTYRVVSVLTVLHQDWLNGKEYKCKVSNKGLPSSIEKTISKAKGQPREPQVYTLPPSQEEMTKNQVSLTCLVKGFYPSDIAVEWESNGQPENNYKTTPPVLDSDGSFFLYSRLTVDKSRWQEGNVFSCSVMHEALHNHYTQKSLSLSLGGGGGSGGGGSGGGGSGGGGSGIPPHVQKSVNNDMIVTDNNGAVKFPQLCKFCDVRFSTCDNQKSCMSNCSITSICEKPQEVCVAVWRKNDENITLETVCHDPKLPYHDFILEDAASPKCIMKEKKKPGETFFMCSCSSDECNDNIIFSEEYNTSNPD

SEQ ID NO: 85 - protein, 214 aa, synthetic construct
  source 1..214: note = LC of anti-HEL and anti-TGFbeta antibody
DIELTQSPATLSVTPGDSVSLSCRASQSISNNLHWYQQKSHESPRLLIKYTSQSMSGIPSRFSGSGSGTDFTLSINSVETEDFGVYFCQQSGSWPRTFGGGTKLDIKRTVAAPSVFIFPPSDEQLKSGTASVVCLLNNFYPREAKVQWKVDNALQSGNSQESVTEQDSKDSTYSLSSTLTLSKADYEKHKVYACEVTHQGLSSPVTKSFNRGEC

SEQ ID NO: 86 - protein, 456 aa, synthetic construct
  source 1..456: note = RG6058(G1DM) HC
EVQLQQSGPGLVKPSQTLSLTCAISGDSVSSNSAAWNWIRQSPSRGLEWLGKTYYRFKWYSDYAVSVKGRITINPDTSKNQFSLQLNSVTPEDTAVFYCTRESTTYDLLAGPFDYWGQGTLVTVSSASTKGPSVFPLAPSSKSTSGGTAALGCLVKDYFPEPVTVSWNSGALTSGVHTFPAVLQSSGLYSLSSVVTVPSSSLGTQTYICNVNHKPSNTKVDKKVEPKSCDKTHTCPPCPAPEAAGGPSVFLFPPKPKDTLMISRTPEVTCVVVDVSHEDPEVKFNWYVDGVEVHNAKTKPREEQYNSTYRVVSVLTVLHQDWLNGKEYKCKVSNKALPAPIEKTISKAKGQPREPQVYTLPPSRDELTKNQVSLTCLVKGFYPSDIAVEWESNGQPENNYKTTPPVLDSDGSFFLYSKLTVDKSRWQQGNVFSCSVMHEALHNHYTQKSLSLSPGK

SEQ ID NO: 87 - protein, 220 aa, synthetic construct; identical to SEQ ID NO: 80
  source 1..220: note = RG6058(G1DM) LC

SEQ ID NO: 88 - protein, 136 aa, synthetic construct
  source 1..136: note = variant of extracellular domain of TGF-betaRII in TF01T
IPPHVQKTVNNDMIVTDNNGAVKFPQLCKFCDVRFSTCDNQKSCMSNCSITSICEKPQEVCVAVWRKNDENITLETVCHDPKLPYHDFILEDAASPKCIMKEKKKPGETFFMCSCSSDECNDNIIFSEEYNTSNPD

SEQ ID NO: 89 - protein, 326 aa, synthetic construct
  source 1..326: note = hIgG4WT CH
ASTKGPSVFPLAPCSRSTSESTAALGCLVKDYFPEPVTVSWNSGALTSGVHTFPAVLQSSGLYSLSSVVTVPSSSLGTKTYTCNVDHKPSNTKVDKRVESKYGPPCPPCPAPEFLGGPSVFLFPPKPKDTLMISRTPEVTCVVVDVSQEDPEVQFNWYVDGVEVHNAKTKPREEQFNSTYRVVSVLTVLHQDWLNGKEYKCKVSNKGLPSSIEKTISKAKGQPREPQVYTLPPSQEEMTKNQVSLTCLVKGFYPSDIAVEWESNGQPENNYKTTPPVLDSDGSFFLYSRLTVDKSRWQEGNVFSCSVMHEALHNHYTQKSLSLSLG

SEQ ID NO: 90 - protein, 330 aa, synthetic construct [sequence omitted]

SEQ ID NO: 91 - protein, 5 aa, synthetic construct
  source 1..5: note = repeat unit in linker
GGGGS

SEQ ID NO: 92 - protein, 6 aa, synthetic construct
  source 1..6: note = fragment in linker
GGGGSG